European Patent Application EP 4 729 070 A1, published April 22, 2026. Title: METHOD OF GENE EDITING USING BASE EDITORS FOR TRANSGENE INSERTION AND MULTIPLEX GENE EDITING. Applicant: Charité. The sequence listing filed with the application follows.

SEQUENCE LISTING (65 sequences)

SEQ ID NO: 1 - DNA, 20 bp, synthetic construct
  source 1..20: mol_type = other DNA
agagtctctcagctggtaca

SEQ ID NO: 2 - DNA, 20 bp, synthetic construct
  source 1..20: mol_type = other DNA
gagaatcaaaatcggtgaat

SEQ ID NO: 3 - DNA, 23 bp, synthetic construct
  source 1..23: mol_type = other DNA
aaagtcagatttgttgctccagg

SEQ ID NO: 4 - DNA, 23 bp, synthetic construct
  source 1..23: mol_type = other DNA
cttacctgggctggggaagaagg

SEQ ID NO: 5 - DNA, 23 bp, synthetic construct
  source 1..23: mol_type = other DNA
agctgcccttacctgggctgggg

SEQ ID NO: 6 - DNA, 23 bp, synthetic construct
  source 1..23: mol_type = other DNA
caccaaagctgcccttacctggg

SEQ ID NO: 7 - DNA, 20 bp, synthetic construct
  source 1..20: mol_type = other DNA
agcccaggtaagggcagctt

SEQ ID NO: 8 - DNA, 20 bp, synthetic construct
  source 1..20: mol_type = other DNA
tgtgctagacatgaggtcta

SEQ ID NO: 9 - DNA, 20 bp, synthetic construct
  source 1..20: mol_type = other DNA
agagcaacagtgctgtggcc

SEQ ID NO: 10 - DNA, 20 bp, synthetic construct
  source 1..20: mol_type = other DNA
aacaaatgtgtcacaaagta

SEQ ID NO: 11 - DNA, 20 bp, synthetic construct
  source 1..20: mol_type = other DNA
gacaccttcttccccagccc

SEQ ID NO: 12 - DNA, 23 bp, synthetic construct
  source 1..23: mol_type = other DNA
ttcttccccagcccaggtaaggg

SEQ ID NO: 13 - DNA, 20 bp, synthetic construct
  source 1..20: mol_type = other DNA
acatccccattaccccaggg

SEQ ID NO: 14 - DNA, 20 bp, synthetic construct
  source 1..20: mol_type = other DNA
tctgtgccaagagataaagc

SEQ ID NO: 15 - DNA, 20 bp, synthetic construct
  source 1..20: mol_type = other DNA
tccagcaggtagcagagttt

SEQ ID NO: 16 - DNA, 20 bp, synthetic construct
  source 1..20: mol_type = other DNA
gaatgacaccatagatgaag

SEQ ID NO: 17 - DNA, 20 bp, synthetic construct
  source 1..20: mol_type = other DNA
tgccttgttcctgagagtga

SEQ ID NO: 18 - DNA, 20 bp, synthetic construct
  source 1..20: mol_type = other DNA
gatggaatcctcttcatcta

SEQ ID NO: 19 - DNA, 20 bp, synthetic construct
  source 1..20: mol_type = other DNA
aggtgggtaccactgggctt

SEQ ID NO: 20 - DNA, 20 bp, synthetic construct
  source 1..20: mol_type = other DNA
gagtgaaggtgggtaccact

SEQ ID NO: 21 - DNA, 20 bp, synthetic construct
  source 1..20: mol_type = other DNA
acaaagtcacatggttcaca

SEQ ID NO: 22 - DNA, 20 bp, synthetic construct
  source 1..20: mol_type = other DNA
cttaccccacttaactatct

SEQ ID NO: 23 - DNA, 20 bp, synthetic construct
  source 1..20: mol_type = other DNA
cttgccccacttaactatct

SEQ ID NO: 24 - DNA, 20 bp, synthetic construct
  source 1..20: mol_type = other DNA
tgggctgtgacaaagtcaca

SEQ ID NO: 25 - DNA, 20 bp, synthetic construct
  source 1..20: mol_type = other DNA
agtcacatggttcacacggc

SEQ ID NO: 26 - DNA, 40 bp, synthetic construct
  source 1..40: mol_type = other DNA
aagctgctttgatataaaaaatctgcatattgggattgtc

SEQ ID NO: 27 - DNA, 20 bp, synthetic construct
  source 1..20: mol_type = other DNA
atctgcatattgggattgtc

SEQ ID NO: 28 - DNA, 20 bp, synthetic construct
  source 1..20: mol_type = other DNA
acagcccaagatagttaagt

SEQ ID NO: 29 - DNA, 20 bp, synthetic construct
  source 1..20: mol_type = other DNA
tttgatataaaaaaggtcta

SEQ ID NO: 30 - DNA, 20 bp, synthetic construct
  source 1..20: mol_type = other DNA
agagtctctcagctggtaca

SEQ ID NO: 31 - DNA, 23 bp, synthetic construct
  source 1..23: mol_type = other DNA
gagtctctcagctggtacacggc

SEQ ID NO: 32 - DNA, 20 bp, synthetic construct
  source 1..20: mol_type = other DNA
gcttacagatcttgccccgc

SEQ ID NO: 33 - DNA, 20 bp, synthetic construct
  source 1..20: mol_type = other DNA
atttacctgaacctctgaat

SEQ ID NO: 34 - DNA, 20 bp, synthetic construct
  source 1..20: mol_type = other DNA
cccttaccaggcttgatgag

SEQ ID NO: 35 - DNA, 20 bp, synthetic construct
  source 1..20: mol_type = other DNA
ctcaccgtctcctggggaga

SEQ ID NO: 36 - DNA, 20 bp, synthetic construct
  source 1..20: mol_type = other DNA
ctcaccggtgtagtgcacca

SEQ ID NO: 37 - DNA, 20 bp, synthetic construct
  source 1..20: mol_type = other DNA
ctactcaccgtctcctgggg

SEQ ID NO: 38 - DNA, 2716 bp, synthetic construct
  source 1..2716: mol_type = other DNA
tttcaggtttccttgagtggcaggccaggcctggccgtgaacgttcactgaaatcatggcctcttggccaagattgatagcttgtgcctgtccctgagtcccagtccatcacgagcagctggtttctaagatgctatttcccgtataaagcatgagaccgtgacttgccagccccacagagccccgcccttgtccatcactggcatctggactccagcctgggttggggcaaagagggaaatgagatcatgtcctaaccctgatcctcttgtcccacagatatccagaaccctgaccctgcctccggatccggagccaccaacttcagcctgctgaagcaggccggcgacgtggaagaaaatcctgggcccatggctcttcctgtgactgcccttctgctgcccctggctctcctgctccatgctgcccggccagacatccagatgacacagacaaccagcagcctcagcgccagcctgggggacagagtgaccattagctgccgggcctctcaggacatcagcaaatacctgaactggtaccagcagaaaccagatggcactgtcaagctgctgatttaccacacctccaggctccacagcggcgtgcccagtcgcttcagcggcagtgggagcgggacagattattccctcacaatctccaacctggagcaggaagatattgccacatacttctgccagcaaggcaacaccctgccatacacatttggaggcggcaccaaattggagatcaccggcggtggtggatctggaggagggggcagcggaggtggcggctctgaggtgaaactgcaggagagtggccctggcctggtggctcccagccagagcctttctgtcacctgcaccgtgtctggggtgtccctgcctgactatggagtctcctggatccggcagcctccaagaaaaggactggaatggctgggcgtcatctggggaagtgagaccacctactataattcagccctcaagtcccggctcaccatcattaaggacaactccaaatcccaggtgttcctgaagatgaattctctccagactgatgacacagccatctactactgtgccaagcattattattacggcgggtcctatgccatggactactggggccaggggaccagtgtcactgtttcttctgaaagcaagtatggccccccatgccctccctgccccggacagccgcgggagccccaggtctacaccctcccaccctccagagatgagctgaccaagaaccaggtttcactgacatgcctggtgaagggcttctacccctctgacattgctgtggagtgggagagcaatgggcagccagagaacaactacaagaccacacctcctgtcctggacagcgacggctccttcttcctctacagtaagctcactgtggacaagagccgctggcagcagggcaatgtcttctcctgcagcgtgatgcacgaggccctgcacaatgcctatacccagaagtcactctctctgagccctggaaagaaggatcccaagttttgggtcctcgtggtggtcgggggtgtgctggcctgctacagcttgctggtcacagtggccttcatcatcttctgggtgcgctccaagaggagccggctgcttcacagtgattacatgaacatgacccccaggaggccaggacccaccaggaagcactaccagccctacgctcccccgcgggactttgctgcttaccgcagcagggtcaaattttctagatctgcagatgcgccggcctatcaacaaggccagaaccagctctataacgagctcaatctaggacgaagagaggagtacgatgttttggacaagagacgtggccgggaccctgagatggggggaaagccgagaaggaagaaccctcaggaaggcctgtacaatgaactgcagaaagataagatggcggaggcctacagtgagattgggatgaaaggcgagcgccggaggggcaaggggcacgatggcctttaccagggtctcagtacagccaccaaggacacctacgacgcccttcacatgcaggccctgccccctcgctaataagaattctaactagagctcgctgatcagcctcgactgtgccttctagttgccagccatctgttgtttgcccctcccccgtgccttccttgaccctggaaggtgccactcccactgtcctttcctaataaaatgaggaaattgcatcgcattgtctgagtaggtgtcattctattctggggggtggggtggggcaggacagcaagggggaggattgggaagagaatagcaggcatgctggggactttggtgccttcgcaggctgtttccttgcttcaggaatggccaggttctgcccagagctctggtcaatgatgtctaaaactcctctgattggtggtctcggccttatccattgccaccaaaaccctctttttactaagaaacagtgagccttgttctggcagtccagagaatgacacgggaaaaaagcagatgaagagaaggtggcaggagagggcacgtggcccagcctcagtctctccaactgagttcctgcctgcctgcctttgctcagactgtttgccccttactgctcttctaggcctcattctaagccccttctccaagttgcctctccttatttctccctgtctgccaaaaaatctttcccagctcactaagtcagtctcacgcagtcactc

SEQ ID NO: 39 - DNA, 2716 bp, synthetic construct
  source 1..2716: mol_type = other DNA
tttcaggtttccttgagtggcaggccaggcctggccgtgaacgttcactgaaatcatggcctcttggccaagattgatagcttgtgcctgtccctgagtcccagtccatcacgagcagctggtttctaagatgctatttcccgtataaagcatgagaccgtgacttgccagccccacagagccccgcccttgtccatcactggcatctggactccagcctgggttggggcaaagagggaaatgagatcatgtcctaaccctgatcctcttgtcccacagatatccagaaccctgaccctgcctccggatccggagccaccaacttcagcctgctgaagcaggccggcgacgtggaagaaaatcctgggcccatggctcttcctgtgactgcccttctgctgcccctggctctcctgctccatgctgcccggccagacatccagatgacacagacaaccagcagcctcagcgccagcctgggggacagagtgaccattagctgccgggcctctcaggacatcagcaaatacctgaactggtaccagcagaaaccagatggcactgtcaagctgctgatttaccacacctccaggctccacagcggcgtgcccagtcgcttcagcggcagtgggagcgggacagattattccctcacaatctccaacctggagcaggaagatattgccacatacttctgccagcaaggcaacaccctgccatacacatttggaggcggcaccaaattggagatcaccggcggtggtggatctggaggagggggcagcggaggtggcggctctgaggtgaaactgcaggagagtggccctggcctggtggctcccagccagagcctttctgtcacctgcaccgtgtctggggtgtccctgcctgactatggagtctcctggatccggcagcctccaagaaaaggactggaatggctgggcgtcatctggggaagtgagaccacctactataattcagccctcaagtcccggctcaccatcattaaggacaactccaaatcccaggtgttcctgaagatgaattctctccagactgatgacacagccatctactactgtgccaagcattattattacggcgggtcctatgccatggactactggggccaggggaccagtgtcactgtttcttctgaaagcaagtatggccccccatgccctccctgccccggacagccgcgggagccccaggtctacaccctcccaccctccagagatgagctgaccaagaaccaggtttcactgacatgcctggtgaagggcttctacccctctgacattgctgtggagtgggagagcaatgggcagccagagaacaactacaagaccacacctcctgtcctggacagcgacggctccttcttcctctacagtaagctcactgtggacaagagccgctggcagcagggcaatgtcttctcctgcagcgtgatgcacgaggccctgcacaatgcctatacccagaagtcactctctctgagccctggaaagaaggatcccaagttttgggtcctcgtggtggtcgggggtgtgctggcctgctacagcttgctggtcacagtggccttcatcatcttctgggtgcgctccaagaggagccggctgcttcacagtgattacatgaacatgacccccaggaggccaggacccaccaggaagcactaccagccctacgctcccccgcgggactttgctgcttaccgcagcagggtcaaattttctagatctgcagatgcgccggcctatcaacaaggccagaaccagctctataacgagctcaatctaggacgaagagaggagtacgatgttttggacaagagacgtggccgggaccctgagatggggggaaagccgagaaggaagaaccctcaggaaggcctgtacaatgaactgcagaaagataagatggcggaggcctacagtgagattgggatgaaaggcgagcgccggaggggcaaggggcacgatggcctttaccagggtctcagtacagccaccaaggacacctacgacgcccttcacatgcaggccctgccccctcgctaataagaattctaactagagctcgctgatcagcctcgactgtgccttctagttgccagccatctgttgtttgcccctcccccgtgccttccttgaccctggaaggtgccactcccactgtcctttcctaataaaatgaggaaattgcatcgcattgtctgagtaggtgtcattctattctggggggtggggtggggcaggacagcaagggggaggattgggaagagaatagcaggcatgctggggactatggacttcaagagcaacagtgctgtggcctggagcaacaaatctgactttgcatgtgcaaacgccttcaacaacagcattattccagaagacaccttcttccccagcccaggtaagggcagctttggtgccttcgcaggctgtttccttgcttcaggaatggccaggttctgcccagagctctggtcaatgatgtctaaaactcctctgattggtggtctcggccttatccattgccaccaaaaccctctttttactaagaaacagtgagccttgttctggcagtccagagaatgacacgggaaaaaagcagatgaagagaaggtggcaggagagggcacgtggcccagcctcagtctctccaactgagttcctgcctgcctgcctttgctcagact

SEQ ID NO: 40 - DNA, 2716 bp, synthetic construct
  source 1..2716: mol_type = other DNA
tttcaggtttccttgagtggcaggccaggcctggccgtgaacgttcactgaaatcatggcctcttggccaagattgatagcttgtgcctgtccctgagtcccagtccatcacgagcagctggtttctaagatgctatttcccgtataaagcatgagaccgtgacttgccagccccacagagccccgcccttgtccatcactggcatctggactccagcctgggttggggcaaagagggaaatgagatcatgtcctaaccctgatcctcttgtcccacagatatccagaaccctgaccctgcctccggatccggagccaccaacttcagcctgctgaagcaggccggcgacgtggaagaaaatcctgggcccatggctcttcctgtgactgcccttctgctgcccctggctctcctgctccatgctgcccggccagacatccagatgacacagacaaccagcagcctcagcgccagcctgggggacagagtgaccattagctgccgggcctctcaggacatcagcaaatacctgaactggtaccagcagaaaccagatggcactgtcaagctgctgatttaccacacctccaggctccacagcggcgtgcccagtcgcttcagcggcagtgggagcgggacagattattccctcacaatctccaacctggagcaggaagatattgccacatacttctgccagcaaggcaacaccctgccatacacatttggaggcggcaccaaattggagatcaccggcggtggtggatctggaggagggggcagcggaggtggcggctctgaggtgaaactgcaggagagtggccctggcctggtggctcccagccagagcctttctgtcacctgcaccgtgtctggggtgtccctgcctgactatggagtctcctggatccggcagcctccaagaaaaggactggaatggctgggcgtcatctggggaagtgagaccacctactataattcagccctcaagtcccggctcaccatcattaaggacaactccaaatcccaggtgttcctgaagatgaattctctccagactgatgacacagccatctactactgtgccaagcattattattacggcgggtcctatgccatggactactggggccaggggaccagtgtcactgtttcttctgaaagcaagtatggccccccatgccctccctgccccggacagccgcgggagccccaggtctacaccctcccaccctccagagatgagctgaccaagaaccaggtttcactgacatgcctggtgaagggcttctacccctctgacattgctgtggagtgggagagcaatgggcagccagagaacaactacaagaccacacctcctgtcctggacagcgacggctccttcttcctctacagtaagctcactgtggacaagagccgctggcagcagggcaatgtcttctcctgcagcgtgatgcacgaggccctgcacaatgcctatacccagaagtcactctctctgagccctggaaagaaggatcccaagttttgggtcctcgtggtggtcgggggtgtgctggcctgctacagcttgctggtcacagtggccttcatcatcttctgggtgcgctccaagaggagccggctgcttcacagtgattacatgaacatgacccccaggaggccaggacccaccaggaagcactaccagccctacgctcccccgcgggactttgctgcttaccgcagcagggtcaaattttctagatctgcagatgcgccggcctatcaacaaggccagaaccagctctataacgagctcaatctaggacgaagagaggagtacgatgttttggacaagagacgtggccgggaccctgagatggggggaaagccgagaaggaagaaccctcaggaaggcctgtacaatgaactgcagaaagataagatggcggaggcctacagtgagattgggatgaaaggcgagcgccggaggggcaaggggcacgatggcctttaccagggtctcagtacagccaccaaggacacctacgacgcccttcacatgcaggccctgccccctcgctaataagaattctaactagagctcgctgatcagcctcgactgtgccttctagttgccagccatctgttgtttgcccctcccccgtgccttccttgaccctggaaggtgccactcccactgtcctttcctaataaaatgaggaaattgcatcgcattgtctgagtaggtgtcattctattctggggggtggggtggggcaggacagcaagggggaggattgggaagagaatagcaggcatgctggggagcctggagcaacaaatctgactttgcatgtgcaaacgccttcaacaacagcattattccagaagacaccttcttccccagcccaggtaagggcagctttggtgccttcgcaggctgtttccttgcttcaggaatggccaggttctgcccagagctctggtcaatgatgtctaaaactcctctgattggtggtctcggccttatccattgccaccaaaaccctctttttactaagaaacagtgagccttgttctggcagtccagagaatgacacgggaaaaaagcagatgaagagaaggtggcaggagagggcacgtggcccagcctcagtctctccaactgagttcctgcctgcctgcctttgctcagactgtttgccccttactgctcttctaggcctc

SEQ ID NO: 41 - DNA, 2683 bp, synthetic construct
  source 1..2683: mol_type = other DNA
tttcaggtttccttgagtggcaggccaggcctggccgtgaacgttcactgaaatcatggcctcttggccaagattgatagcttgtgcctgtccctgagtcccagtccatcacgagcagctggtttctaagatgctatttcccgtataaagcatgagaccgtgacttgccagccccacagagccccgcccttgtccatcactggcatctggactccagcctgggttggggcaaagagggaaatgagatcatgtcctaaccctgatcctcttgtcccacagatatccagaaccctgaccctgcctccggatccggagccaccaacttcagcctgctgaagcaggccggcgacgtggaagaaaatcctgggcccatggctcttcctgtgactgcccttctgctgcccctggctctcctgctccatgctgcccggccagacatccagatgacacagacaaccagcagcctcagcgccagcctgggggacagagtgaccattagctgccgggcctctcaggacatcagcaaatacctgaactggtaccagcagaaaccagatggcactgtcaagctgctgatttaccacacctccaggctccacagcggcgtgcccagtcgcttcagcggcagtgggagcgggacagattattccctcacaatctccaacctggagcaggaagatattgccacatacttctgccagcaaggcaacaccctgccatacacatttggaggcggcaccaaattggagatcaccggcggtggtggatctggaggagggggcagcggaggtggcggctctgaggtgaaactgcaggagagtggccctggcctggtggctcccagccagagcctttctgtcacctgcaccgtgtctggggtgtccctgcctgactatggagtctcctggatccggcagcctccaagaaaaggactggaatggctgggcgtcatctggggaagtgagaccacctactataattcagccctcaagtcccggctcaccatcattaaggacaactccaaatcccaggtgttcctgaagatgaattctctccagactgatgacacagccatctactactgtgccaagcattattattacggcgggtcctatgccatggactactggggccaggggaccagtgtcactgtttcttctgaaagcaagtatggccccccatgccctccctgccccggacagccgcgggagccccaggtctacaccctcccaccctccagagatgagctgaccaagaaccaggtttcactgacatgcctggtgaagggcttctacccctctgacattgctgtggagtgggagagcaatgggcagccagagaacaactacaagaccacacctcctgtcctggacagcgacggctccttcttcctctacagtaagctcactgtggacaagagccgctggcagcagggcaatgtcttctcctgcagcgtgatgcacgaggccctgcacaatgcctatacccagaagtcactctctctgagccctggaaagaaggatcccaagttttgggtcctcgtggtggtcgggggtgtgctggcctgctacagcttgctggtcacagtggccttcatcatcttctgggtgcgctccaagaggagccggctgcttcacagtgattacatgaacatgacccccaggaggccaggacccaccaggaagcactaccagccctacgctcccccgcgggactttgctgcttaccgcagcagggtcaaattttctagatctgcagatgcgccggcctatcaacaaggccagaaccagctctataacgagctcaatctaggacgaagagaggagtacgatgttttggacaagagacgtggccgggaccctgagatggggggaaagccgagaaggaagaaccctcaggaaggcctgtacaatgaactgcagaaagataagatggcggaggcctacagtgagattgggatgaaaggcgagcgccggaggggcaaggggcacgatggcctttaccagggtctcagtacagccaccaaggacacctacgacgcccttcacatgcaggccctgccccctcgctaataagaattctaactagagctcgctgatcagcctcgactgtgccttctagttgccagccatctgttgtttgcccctcccccgtgccttccttgaccctggaaggtgccactcccactgtcctttcctaataaaatgaggaaattgcatcgcattgtctgagtaggtgtcattctattctggggggtggggtggggcaggacagcaagggggaggattgggaagagaatagcaggcatgctggggaaaggattctgatgtgtatatcacagacaaaactgtgctagacatgaggtctatggacttcaagagcaacagtgctgtggcctggagcaacaaatctgactttgcatgtgcaaacgccttcaacaacagcattattccagaagacaccttcttccccagcccaggtaagggcagctttggtgccttcgcaggctgtttccttgcttcaggaatggccaggttctgcccagagctctggtcaatgatgtctaaaactcctctgattggtggtctcggccttatccattgccaccaaaaccctctttttactaagaaacagtgagccttgttctggcagtccagagaatgacacgggaaaaaagcagatg

SEQ ID NO: 42 - DNA, 2716 bp, synthetic construct; identical to SEQ ID NO: 38
  source 1..2716: mol_type = other DNA

SEQ ID NO: 43 - DNA, 2716 bp, synthetic construct; identical to SEQ ID NO: 38
  source 1..2716: mol_type = other DNA

SEQ ID NO: 44 - DNA, 2802 bp, synthetic construct
  source 1..2802: mol_type = other DNA
cctattaaataaaagaataagcagtattattaagtagccctgcatttcaggtttccttgagtggcaggccaggcctggccgtgaacgttcactgaaatcatggcctcttggccaagattgatagcttgtgcctgtccctgagtcccagtccatcacgagcagctggtttctaagatgctatttcccgtataaagcatgagaccgtgacttgccagccccacagagccccgcccttgtccatcactggcatctggactccagcctgggttggggcaaagagggaaatgagatcatgtcctaaccctgatcctcttgtcccacagatatccagaaccctgaccctgccgtgtaccagctgagagactctaaatccagtgacaagtctgtctgcctattcaccgccaccaacttctctcttttgaagcaggccggagatgtggaagaaaatcctgggcccatggctcttcctgtgactgcccttctgctgcccctggctctcctgctccatgctgcccggccagacatccagatgacacagacaaccagcagcctcagcgccagcctgggggacagagtgaccattagctgccgggcctctcaggacatcagcaaatacctgaactggtaccagcagaaaccagatggcactgtcaagctgctgatttaccacacctccaggctccacagcggcgtgcccagtcgcttcagcggcagtgggagcgggacagattattccctcacaatctccaacctggagcaggaagatattgccacatacttctgccagcaaggcaacaccctgccatacacatttggaggcggcaccaaattggagatcaccggcggtggtggatctggaggagggggcagcggaggtggcggctctgaggtgaaactgcaggagagtggccctggcctggtggctcccagccagagcctttctgtcacctgcaccgtgtctggggtgtccctgcctgactatggagtctcctggatccggcagcctccaagaaaaggactggaatggctgggcgtcatctggggaagtgagaccacctactataattcagccctcaagtcccggctcaccatcattaaggacaactccaaatcccaggtgttcctgaagatgaattctctccagactgatgacacagccatctactactgtgccaagcattattattacggcgggtcctatgccatggactactggggccaggggaccagtgtcactgtttcttctgaaagcaagtatggccccccatgccctccctgccccggacagccgcgggagccccaggtctacaccctcccaccctccagagatgagctgaccaagaaccaggtttcactgacatgcctggtgaagggcttctacccctctgacattgctgtggagtgggagagcaatgggcagccagagaacaactacaagaccacacctcctgtcctggacagcgacggctccttcttcctctacagtaagctcactgtggacaagagccgctggcagcagggcaatgtcttctcctgcagcgtgatgcacgaggccctgcacaatgcctatacccagaagtcactctctctgagccctggaaagaaggatcccaagttttgggtcctcgtggtggtcgggggtgtgctggcctgctacagcttgctggtcacagtggccttcatcatcttctgggtgcgctccaagaggagccggctgcttcacagtgattacatgaacatgacccccaggaggccaggacccaccaggaagcactaccagccctacgctcccccgcgggactttgctgcttaccgcagcagggtcaaattttctagatctgcagatgcgccggcctatcaacaaggccagaaccagctctataacgagctcaatctaggacgaagagaggagtacgatgttttggacaagagacgtggccgggaccctgagatggggggaaagccgagaaggaagaaccctcaggaaggcctgtacaatgaactgcagaaagataagatggcggaggcctacagtgagattgggatgaaaggcgagcgccggaggggcaaggggcacgatggcctttaccagggtctcagtacagccaccaaggacacctacgacgcccttcacatgcaggccctgccccctcgctaataagaattctaactagagctcgctgatcagcctcgactgtgccttctagttgccagccatctgttgtttgcccctcccccgtgccttccttgaccctggaaggtgccactcccactgtcctttcctaataaaatgaggaaattgcatcgcattgtctgagtaggtgtcattctattctggggggtggggtggggcaggacagcaagggggaggattgggaagagaatagcaggcatgctggggactatggacttcaagagcaacagtgctgtggcctggagcaacaaatctgactttgcatgtgcaaacgccttcaacaacagcattattccagaagacaccttcttccccagcccaggtaagggcagctttggtgccttcgcaggctgtttccttgcttcaggaatggccaggttctgcccagagctctggtcaatgatgtctaaaactcctctgattggtggtctcggccttatccattgccaccaaaaccctctttttactaagaaacagtgagccttgttctggcagtccagagaatgacacgggaaaaaagcagatgaagagaaggtggcaggagagggcacgtggcccagcctcagtctctccaactgagttcctgcctgcctgcctttgctcagact

SEQ ID NO: 45 - DNA, 2802 bp, synthetic construct
  source 1..2802: mol_type = other DNA
cctattaaataaaagaataagcagtattattaagtagccctgcatttcaggtttccttgagtggcaggccaggcctggccgtgaacgttcactgaaatcatggcctcttggccaagattgatagcttgtgcctgtccctgagtcccagtccatcacgagcagctggtttctaagatgctatttcccgtataaagcatgagaccgtgacttgccagccccacagagccccgcccttgtccatcactggcatctggactccagcctgggttggggcaaagagggaaatgagatcatgtcctaaccctgatcctcttgtcccacagatatccagaaccctgaccctgccgtgtaccagctgagagactctaaatccagtgacaagtctgtctgcctattcaccgccaccaacttctctcttttgaagcaggccggagatgtggaagaaaatcctgggcccatggctcttcctgtgactgcccttctgctgcccctggctctcctgctccatgctgcccggccagacatccagatgacacagacaaccagcagcctcagcgccagcctgggggacagagtgaccattagctgccgggcctctcaggacatcagcaaatacctgaactggtaccagcagaaaccagatggcactgtcaagctgctgatttaccacacctccaggctccacagcggcgtgcccagtcgcttcagcggcagtgggagcgggacagattattccctcacaatctccaacctggagcaggaagatattgccacatacttctgccagcaaggcaacaccctgccatacacatttggaggcggcaccaaattggagatcaccggcggtggtggatctggaggagggggcagcggaggtggcggctctgaggtgaaactgcaggagagtggccctggcctggtggctcccagccagagcctttctgtcacctgcaccgtgtctggggtgtccctgcctgactatggagtctcctggatccggcagcctccaagaaaaggactggaatggctgggcgtcatctggggaagtgagaccacctactataattcagccctcaagtcccggctcaccatcattaaggacaactccaaatcccaggtgttcctgaagatgaattctctccagactgatgacacagccatctactactgtgccaagcattattattacggcgggtcctatgccatggactactggggccaggggaccagtgtcactgtttcttctgaaagcaagtatggccccccatgccctccctgccccggacagccgcgggagccccaggtctacaccctcccaccctccagagatgagctgaccaagaaccaggtttcactgacatgcctggtgaagggcttctacccctctgacattgctgtggagtgggagagcaatgggcagccagagaacaactacaagaccacacctcctgtcctggacagcgacggctccttcttcctctacagtaagctcactgtggacaagagccgctggcagcagggcaatgtcttctcctgcagcgtgatgcacgaggccctgcacaatgcctatacccagaagtcactctctctgagccctggaaagaaggatcccaagttttgggtcctcgtggtggtcgggggtgtgctggcctgctacagcttgctggtcacagtggccttcatcatcttctgggtgcgctccaagaggagccggctgcttcacagtgattacatgaacatgacccccaggaggccaggacccaccaggaagcactaccagccctacgctcccccgcgggactttgctgcttaccgcagcagggtcaaattttctagatctgcagatgcgccggcctatcaacaaggccagaaccagctctataacgagctcaatctaggacgaagagaggagtacgatgttttggacaagagacgtggccgggaccctgagatggggggaaagccgagaaggaagaaccctcaggaaggcctgtacaatgaactgcagaaagataagatggcggaggcctacagtgagattgggatgaaaggcgagcgccggaggggcaaggggcacgatggcctttaccagggtctcagtacagccaccaaggacacctacgacgcccttcacatgcaggccctgccccctcgctaataagaattctaactagagctcgctgatcagcctcgactgtgccttctagttgccagccatctgttgtttgcccctcccccgtgccttccttgaccctggaaggtgccactcccactgtcctttcctaataaaatgaggaaattgcatcgcattgtctgagtaggtgtcattctattctggggggtggggtggggcaggacagcaagggggaggattgggaagagaatagcaggcatgctggggagcctggagcaacaaatctgactttgcatgtgcaaacgccttcaacaacagcattattccagaagacaccttcttccccagcccaggtaagggcagctttggtgccttcgcaggctgtttccttgcttcaggaatggccaggttctgcccagagctctggtcaatgatgtctaaaactcctctgattggtggtctcggccttatccattgccaccaaaaccctctttttactaagaaacagtgagccttgttctggcagtccagagaatgacacgggaaaaaagcagatgaagagaaggtggcaggagagggcacgtggcccagcctcagtctctccaactgagttcctgcctgcctgcctttgctcagactgtttgccccttactgctcttctaggcctc

SEQ ID NO: 46 - DNA, 2769 bp, synthetic construct
  source 1..2769: mol_type = other DNA
cctattaaataaaagaataagcagtattattaagtagccctgcatttcaggtttccttgagtggcaggccaggcctggccgtgaacgttcactgaaatcatggcctcttggccaagattgatagcttgtgcctgtccctgagtcccagtccatcacgagcagctggtttctaagatgctatttcccgtataaagcatgagaccgtgacttgccagccccacagagccccgcccttgtccatcactggcatctggactccagcctgggttggggcaaagagggaaatgagatcatgtcctaaccctgatcctcttgtcccacagatatccagaaccctgaccctgccgtgtaccagctgagagactctaaatccagtgacaagtctgtctgcctattcaccgccaccaacttctctcttttgaagcaggccggagatgtggaagaaaatcctgggcccatggctcttcctgtgactgcccttctgctgcccctggctctcctgctccatgctgcccggccagacatccagatgacacagacaaccagcagcctcagcgccagcctgggggacagagtgaccattagctgccgggcctctcaggacatcagcaaatacctgaactggtaccagcagaaaccagatggcactgtcaagctgctgatttaccacacctccaggctccacagcggcgtgcccagtcgcttcagcggcagtgggagcgggacagattattccctcacaatctccaacctggagcaggaagatattgccacatacttctgccagcaaggcaacaccctgccatacacatttggaggcggcaccaaattggagatcaccggcggtggtggatctggaggagggggcagcggaggtggcggctctgaggtgaaactgcaggagagtggccctggcctggtggctcccagccagagcctttctgtcacctgcaccgtgtctggggtgtccctgcctgactatggagtctcctggatccggcagcctccaagaaaaggactggaatggctgggcgtcatctggggaagtgagaccacctactataattcagccctcaagtcccggctcaccatcattaaggacaactccaaatcccaggtgttcctgaagatgaattctctccagactgatgacacagccatctactactgtgccaagcattattattacggcgggtcctatgccatggactactggggccaggggaccagtgtcactgtttcttctgaaagcaagtatggccccccatgccctccctgccccggacagccgcgggagccccaggtctacaccctcccaccctccagagatgagctgaccaagaaccaggtttcactgacatgcctggtgaagggcttctacccctctgacattgctgtggagtgggagagcaatgggcagccagagaacaactacaagaccacacctcctgtcctggacagcgacggctccttcttcctctacagtaagctcactgtggacaagagccgctggcagcagggcaatgtcttctcctgcagcgtgatgcacgaggccctgcacaatgcctatacccagaagtcactctctctgagccctggaaagaaggatcccaagttttgggtcctcgtggtggtcgggggtgtgctggcctgctacagcttgctggtcacagtggccttcatcatcttctgggtgcgctccaagaggagccggctgcttcacagtgattacatgaacatgacccccaggaggccaggacccaccaggaagcactaccagccctacgctcccccgcgggactttgctgcttaccgcagcagggtcaaattttctagatctgcagatgcgccggcctatcaacaaggccagaaccagctctataacgagctcaatctaggacgaagagaggagtacgatgttttggacaagagacgtggccgggaccctgagatggggggaaagccgagaaggaagaaccctcaggaaggcctgtacaatgaactgcagaaagataagatggcggaggcctacagtgagattgggatgaaaggcgagcgccggaggggcaaggggcacgatggcctttaccagggtctcagtacagccaccaaggacacctacgacgcccttcacatgcaggccctgccccctcgctaataagaattctaactagagctcgctgatcagcctcgactgtgccttctagttgccagccatctgttgtttgcccctcccccgtgccttccttgaccctggaaggtgccactcccactgtcctttcctaataaaatgaggaaattgcatcgcattgtctgagtaggtgtcattctattctggggggtggggtggggcaggacagcaagggggaggattgggaagagaatagcaggcatgctggggaaaggattctgatgtgtatatcacagacaaaactgtgctagacatgaggtctatggacttcaagagcaacagtgctgtggcctggagcaacaaatctgactttgcatgtgcaaacgccttcaacaacagcattattccagaagacaccttcttccccagcccaggtaagggcagctttggtgccttcgcaggctgtttccttgcttcaggaatggccaggttctgcccagagctctggtcaatgatgtctaaaactcctctgattggtggtctcggccttatccattgccaccaaaaccctctttttactaagaaacagtgagccttgttctggcagtccagagaatgacacgggaaaaaagcagatg

SEQ ID NO: 47 - DNA, 2822 bp, synthetic construct
  source 1..2822: mol_type = other DNA
tgatagcttgtgcctgtccctgagtcccagtccatcacgagcagctggtttctaagatgctatttcccgtataaagcatgagaccgtgacttgccagccccacagagccccgcccttgtccatcactggcatctggactccagcctgggttggggcaaagagggaaatgagatcatgtcctaaccctgatcctcttgtcccacagatatccagaaccctgaccctgccgtgtaccagctgagagactctaaatccagtgacaagtctgtctgcctattcaccgattttgattctcaaacaaatgtgtcacaaagtaaggattctgatgtgtatatcacagacaaaactgtgctagacatgaggtctatggacttcaagagcaacagtgctgtggcctggagcggatccggagccaccaacttcagcctgctgaagcaggccggcgacgtggaagaaaatcctgggcccatggctcttcctgtgactgcccttctgctgcccctggctctcctgctccatgctgcccggccagacatccagatgacacagacaaccagcagcctcagcgccagcctgggggacagagtgaccattagctgccgggcctctcaggacatcagcaaatacctgaactggtaccagcagaaaccagatggcactgtcaagctgctgatttaccacacctccaggctccacagcggcgtgcccagtcgcttcagcggcagtgggagcgggacagattattccctcacaatctccaacctggagcaggaagatattgccacatacttctgccagcaaggcaacaccctgccatacacatttggaggcggcaccaaattggagatcaccggcggtggtggatctggaggagggggcagcggaggtggcggctctgaggtgaaactgcaggagagtggccctggcctggtggctcccagccagagcctttctgtcacctgcaccgtgtctggggtgtccctgcctgactatggagtctcctggatccggcagcctccaagaaaaggactggaatggctgggcgtcatctggggaagtgagaccacctactataattcagccctcaagtcccggctcaccatcattaaggacaactccaaatcccaggtgttcctgaagatgaattctctccagactgatgacacagccatctactactgtgccaagcattattattacggcgggtcctatgccatggactactggggccaggggaccagtgtcactgtttcttctgaaagcaagtatggccccccatgccctccctgccccggacagccgcgggagccccaggtctacaccctcccaccctccagagatgagctgaccaagaaccaggtttcactgacatgcctggtgaagggcttctacccctctgacattgctgtggagtgggagagcaatgggcagccagagaacaactacaagaccacacctcctgtcctggacagcgacggctccttcttcctctacagtaagctcactgtggacaagagccgctggcagcagggcaatgtcttctcctgcagcgtgatgcacgaggccctgcacaatgcctatacccagaagtcactctctctgagccctggaaagaaggatcccaagttttgggtcctcgtggtggtcgggggtgtgctggcctgctacagcttgctggtcacagtggccttcatcatcttctgggtgcgctccaagaggagccggctgcttcacagtgattacatgaacatgacccccaggaggccaggacccaccaggaagcactaccagccctacgctcccccgcgggactttgctgcttaccgcagcagggtcaaattttctagatctgcagatgcgccggcctatcaacaaggccagaaccagctctataacgagctcaatctaggacgaagagaggagtacgatgttttggacaagagacgtggccgggaccctgagatggggggaaagccgagaaggaagaaccctcaggaaggcctgtacaatgaactgcagaaagataagatggcggaggcctacagtgagattgggatgaaaggcgagcgccggaggggcaaggggcacgatggcctttaccagggtctcagtacagccaccaaggacacctacgacgcccttcacatgcaggccctgccccctcgctaataagaattctaactagagctcgctgatcagcctcgactgtgccttctagttgccagccatctgttgtttgcccctcccccgtgccttccttgaccctggaaggtgccactcccactgtcctttcctaataaaatgaggaaattgcatcgcattgtctgagtaggtgtcattctattctggggggtggggtggggcaggacagcaagggggaggattgggaagagaatagcaggcatgctggggataagggcagctttggtgccttcgcaggctgtttccttgcttcaggaatggccaggttctgcccagagctctggtcaatgatgtctaaaactcctctgattggtggtctcggccttatccattgccaccaaaaccctctttttactaagaaacagtgagccttgttctggcagtccagagaatgacacgggaaaaaagcagatgaagagaaggtggcaggagagggcacgtggcccagcctcagtctctccaactgagttcctgcctgcctgcctttgctcagactgtttgccccttactgctcttctaggcctcattctaagccccttctccaagttgcctctccttatttctccctgtctgccaaaaaatctttcccagctcactaagtcagtctcacgcagtcactc

SEQ ID NO: 48 - DNA, 2301 bp, synthetic construct
  source 1..2301: mol_type = other DNA
atctcatttgaccatcatttgacctattgtctccctgtgggtaggcctcagagccacacacctcaggccaggagtaccattcatccagacgtgaacatcttcccgaggcttccagagttcttggttcacaccggggctaacatggctgggcttctgctgcagtggcaggagctctgtgcacagagaacagcctcatctgctcgccttgtttccacctcccctcccattgccccaggttctttggccccacagcggccacatctgccgttggtgccaataggttttccaggagctggttgaggtgggagggagggagagggttgtgatcaggctgaggcatggggattggatatagtctccgtgtcatgatttatttggtcagtcagtcctagtgcgaccctggggtaatggggatgtgttctcgtcacgttgggcctggctgaccagctttatctcttggcacagaggcaggcagcggcgctaccaatttttctttgttgaagcaggccggggatgtggaggaaaatccggggccaatggctcttcctgtgactgcccttctgctgcccctggctctcctgctccatgctgcccggccagacatccagatgacacagacaaccagcagcctcagcgccagcctgggggacagagtgaccattagctgccgggcctctcaggacatcagcaaatacctgaactggtaccagcagaaaccagatggcactgtcaagctgctgatttaccacacctccaggctccacagcggcgtgcccagtcgcttcagcggcagtgggagcgggacagattattccctcacaatctccaacctggagcaggaagatattgccacatacttctgccagcaaggcaacaccctgccatacacatttggaggcggcaccaaattggagatcaccggcggtggtggatctggaggagggggcagcggaggtggcggctctgaggtgaaactgcaggagagtggccctggcctggtggctcccagccagagcctttctgtcacctgcaccgtgtctggggtgtccctgcctgactatggagtctcctggatccggcagcctccaagaaaaggactggaatggctgggcgtcatctggggaagtgagaccacctactataattcagccctcaagtcccggctcaccatcattaaggacaactccaaatcccaggtgttcctgaagatgaattctctccagactgatgacacagccatctactactgtgccaagcattattattacggcgggtcctatgccatggactactggggccaggggaccagtgtcactgtttcttctgaaagcaagtatggccccccatgccctccctgccccggacagccgcgggagccccaggtctacaccctcccaccctccagagatgagctgaccaagaaccaggtttcactgacatgcctggtgaagggcttctacccctctgacattgctgtggagtgggagagcaatgggcagccagagaacaactacaagaccacacctcctgtcctggacagcgacggctccttcttcctctacagtaagctcactgtggacaagagccgctggcagcagggcaatgtcttctcctgcagcgtgatgcacgaggccctgcacaatgcctatacccagaagtcactctctctgagccctggaaagaaggatcccaagttttgggtcctcgtggtggtcgggggtgtgctggcctgctacagcttgctggtcacagtggccttcatcatcttctgggtgcgctccaagaggagccggctgcttcacagtgattacatgaacatgacccccaggaggccaggacccaccaggaagcactaccagccctacgctcccccgcgggactttgctgcttaccgcagcagagtgaaggtgggtaccactgggctttgggaggagggcacggggtcccccacttgatggatgttcagaggggccttggtcttggaaggtctcaagctcgggtggtgcctggggcttggtatccaggagcaaagcaaggaccagccaagtgtgtgccttgagtgggctgaggaggaggtggcagtgtctggctgagatggacagggtaggagggagagcctggtgctaggcacctccatgacaagccgtacaaatgtgtgcacatcagagtgtcccagggaaggcgatgctactggtgacaaaggggcttacactcaggcagaggtccttctttccaagtgtgaatgaaggccatgttagcctttctcttgaaaaggccctttcctcatctgtaactggggag

SEQ ID NO: 49 - DNA, 2301 bp, synthetic construct; identical to SEQ ID NO: 48
  source 1..2301: mol_type = other DNA

SEQ ID NO: 50 - DNA, 2231 bp, synthetic construct
  source 1..2231: mol_type = other DNA
tcttcccgaggcttccagagttcttggttcacaccggggctaacatggctgggcttctgctgcagtggcaggagctctgtgcacagagaacagcctcatctgctcgccttgtttccacctcccctcccattgccccaggttctttggccccacagcggccacatctgccgttggtgccaataggttttccaggagctggttgaggtgggagggagggagagggttgtgatcaggctgaggcatggggattggatatagtctccgtgtcatgatttatttggtcagtcagtcctagtgccaccctggggtaatggggatgtgttctcgtcaccttgggcctggctgaccagctttatctcttggcacagaggcacagagctttggcctgctggatcccaaaggcagcggcgctaccaatttttctttgttgaagcaggccggggatgtggaggaaaatccggggccaatggctcttcctgtgactgcccttctgctgcccctggctctcctgctccatgctgcccggccagacatccagatgacacagacaaccagcagcctcagcgccagcctgggggacagagtgaccattagctgccgggcctctcaggacatcagcaaatacctgaactggtaccagcagaaaccagatggcactgtcaagctgctgatttaccacacctccaggctccacagcggcgtgcccagtcgcttcagcggcagtgggagcgggacagattattccctcacaatctccaacctggagcaggaagatattgccacatacttctgccagcaaggcaacaccctgccatacacatttggaggcggcaccaaattggagatcaccggcggtggtggatctggaggagggggcagcggaggtggcggctctgaggtgaaactgcaggagagtggccctggcctggtggctcccagccagagcctttctgtcacctgcaccgtgtctggggtgtccctgcctgactatggagtctcctggatccggcagcctccaagaaaaggactggaatggctgggcgtcatctggggaagtgagaccacctactataattcagccctcaagtcccggctcaccatcattaaggacaactccaaatcccaggtgttcctgaagatgaattctctccagactgatgacacagccatctactactgtgccaagcattattattacggcgggtcctatgccatggactactggggccaggggaccagtgtcactgtttcttctgaaagcaagtatggccccccatgccctccctgccccggacagccgcgggagccccaggtctacaccctcccaccctccagagatgagctgaccaagaaccaggtttcactgacatgcctggtgaagggcttctacccctctgacattgctgtggagtgggagagcaatgggcagccagagaacaactacaagaccacacctcctgtcctggacagcgacggctccttcttcctctacagtaagctcactgtggacaagagccgctggcagcagggcaatgtcttctcctgcagcgtgatgcacgaggccctgcacaatgcctatacccagaagtcactctctctgagccctggaaagaaggatcccaagttttgggtcctcgtggtggtcgggggtgtgctggcctgctacagcttgctggtcacagtggccttcatcatcttctgggtgcgctccaagaggagccggctgcttcacagtgattacatgaacatgacccccaggaggccaggacccaccaggaagcactaccagccctacgctcccccgcgggactttgctgcttaccgcagcagagtgaaggtgggtaccactgggctttgggaggagggcacggggtcccccacttgatggatgttcagaggggccttggtcttggaaggtctcaagctcgggtggtgcctggggcttggtatccaggagcaaagcaaggaccagccaagtgtgtgccttgagtgggctgaggaggaggtggcagtgtctggctgagatggacagggtaggagggagagcctggtgctaggcacctccatgacaagccgtacaaatgtgtgcacatcagagtgtcccagggaaggcgatgctactggtgacaaaggggcttacactcaggcagaggtccttctttccaagtgtgaatgaaggccatgttagcctttctcttgaaaaggccctttcctcatctgtaactggggag

SEQ ID NO: 51 - DNA, 2231 bp, synthetic construct; identical to SEQ ID NO: 50
  source 1..2231: mol_type = other DNA

SEQ ID NO: 52 - DNA, 2231 bp, synthetic construct
  source 1..2231: mol_type = other DNA
tcttcccgaggcttccagagttcttggttcacaccggggctaacatggctgggcttctgctgcagtggcaggagctctgtgcacagagaacagcctcatctgctcgccttgtttccacctcccctcccattgccccaggttctttggccccacagcggccacatctgccgttggtgccaataggttttccaggagctggttgaggtgggagggagggagagggttgtgatcaggctgaggcatggggattggatatagtctccgtgtcatgatttatttggtcagtcagtcctagtgccaccctggggtaatggggatgtgttctcgtcaccttgggcctggctgaccagctttatctcttggcacagaggcacagagctttggcctgctggatcccaaaggcagcggcgctaccaatttttctttgttgaagcaggccggggatgtggaggaaaatccggggccaatggctcttcctgtgactgcccttctgctgcccctggctctcctgctccatgctgcccggccagacatccagatgacacagacaaccagcagcctcagcgccagcctgggggacagagtgaccattagctgccgggcctctcaggacatcagcaaatacctgaactggtaccagcagaaaccagatggcactgtcaagctgctgatttaccacacctccaggctccacagcggcgtgcccagtcgcttcagcggcagtgggagcgggacagattattccctcacaatctccaacctggagcaggaagatattgccacatacttctgccagcaaggcaacaccctgccatacacatttggaggcggcaccaaattggagatcaccggcggtggtggatctggaggagggggcagcggaggtggcggctctgaggtgaaactgcaggagagtggccctggcctggtggctcccagccagagcctttctgtcacctgcaccgtgtctggggtgtccctgcctgactatggagtctcctggatccggcagcctccaagaaaaggactggaatggctgggcgtcatctggggaagtgagaccacctactataattcagccctcaagtcccggctcaccatcattaaggacaactccaaatcccaggtgttcctgaagatgaattctctccagactgatgacacagccatctactactgtgccaagcattattattacggcgggtcctatgccatggactactggggccaggggaccagtgtcactgtttcttctgaaagcaagtatggccccccatgccctccctgccccggacagccgcgggagccccaggtctacaccctcccaccctccagagatgagctgaccaagaaccaggtttcactgacatgcctggtgaagggcttctacccctctgacattgctgtggagtgggagagcaatgggcagccagagaacaactacaagaccacacctcctgtcctggacagcgacggctccttcttcctctacagtaagctcactgtggacaagagccgctggcagcagggcaatgtcttctcctgcagcgtgatgcacgaggccctgcacaatgcctatacccagaagtcactctctctgagccctggaaagaaggatcccaagttttgggtcctcgtggtggtcgggggtgtgctggcctgctacagcttgctggtcacagtggccttcatcatcttctgggtgcgctccaagaggagccggctgcttcacagtgattacatgaacatgacccccaggaggccaggacccaccaggaagcactaccagccctacgctcccccgcgggactttgctgcttaccgcagcagagtgaaggtgggtaccactgcgctttgcgaggagggcacggggtcccccacttgatggatgttcagaggggccttggtcttggaaggtctcaagctcgggtggtgcctggggcttggtatccaggagcaaagcaaggaccagccaagtgtgtgccttgagtgggctgaggaggaggtggcagtgtctggctgagatggacagggtaggagggagagcctggtgctaggcacctccatgacaagccgtacaaatgtgtgcacatcagagtgtcccagggaaggcgatgctactggtgacaaaggggcttacactcaggcagaggtccttctttccaagtgtgaatgaaggccatgttagcctttctcttgaaaaggccctttcctcatctgtaactggggag

SEQ ID NO: 53 - DNA, 2231 bp, synthetic construct; identical to SEQ ID NO: 52
  source 1..2231: mol_type = other DNA

SEQ ID NO: 54 - DNA, 2231 bp, synthetic construct
  source 1..2231: mol_type = other DNA
acaccggggctaacatggctgggcttctgctgcagtggcaggagctctgtgcacagagaacagcctcatctgctcgccttgtttccacctcccctcccattgccccaggttctttggccccacagcggccacatctgccgttggtgccaataggttttccaggagctggttgaggtgggagggagggagagggttgtgatcaggctgaggcatggggattggatatagtctccgtgtcatgatttatttggtcagtcagtcctagtgccaccctggggtaatggggatgtgttctcgtcaccttgggcctggctgaccagctttatctcttggcacagaggcacagagctttggcctgctggatctcaaactctgctacctgctggatggaatcctcttcggcagcggcgctaccaatttttctttgttgaagcaggccggggatgtggaggaaaatccggggccaatggctcttcctgtgactgcccttctgctgcccctggctctcctgctccatgctgcccggccagacatccagatgacacagacaaccagcagcctcagcgccagcctgggggacagagtgaccattagctgccgggcctctcaggacatcagcaaatacctgaactggtaccagcagaaaccagatggcactgtcaagctgctgatttaccacacctccaggctccacagcggcgtgcccagtcgcttcagcggcagtgggagcgggacagattattccctcacaatctccaacctggagcaggaagatattgccacatacttctgccagcaaggcaacaccctgccatacacatttggaggcggcaccaaattggagatcaccggcggtggtggatctggaggagggggcagcggaggtggcggctctgaggtgaaactgcaggagagtggccctggcctggtggctcccagccagagcctttctgtcacctgcaccgtgtctggggtgtccctgcctgactatggagtctcctggatccggcagcctccaagaaaaggactggaatggctgggcgtcatctggggaagtgagaccacctactataattcagccctcaagtcccggctcaccatcattaaggacaactccaaatcccaggtgttcctgaagatgaattctctccagactgatgacacagccatctactactgtgccaagcattattattacggcgggtcctatgccatggactactggggccaggggaccagtgtcactgtttcttctgaaagcaagtatggccccccatgccctccctgccccggacagccgcgggagccccaggtctacaccctcccaccctccagagatgagctgaccaagaaccaggtttcactgacatgcctggtgaagggcttctacccctctgacattgctgtggagtgggagagcaatgggcagccagagaacaactacaagaccacacctcctgtcctggacagcgacggctccttcttcctctacagtaagctcactgtggacaagagccgctggcagcagggcaatgtcttctcctgcagcgtgatgcacgaggccctgcacaatgcctatacccagaagtcactctctctgagccctggaaagaaggatcccaagttttgggtcctcgtggtggtcgggggtgtgctggcctgctacagcttgctggtcacagtggccttcatcatcttctgggtgcgctccaagaggagccggctgcttcacagtgattacatgaacatgacccccaggaggccaggacccaccaggaagcactaccagccctacgctcccccgcgggactttgctgcttaccgcagcagagtgaaggtgggtaccactgggctttgggaggagggcacggggtcccccacttgatggatgttcagaggggccttggtcttggaaggtctcaagctcgggtggtgcctggggcttggtatccaggagcaaagcaaggaccagccaagtgtgtgccttgagtgggctgaggaggaggtggcagtgtctggctgagatggacagggtaggagggagagcctggtgctaggcacctccatgacaagccgtacaaatgtgtgcacatcagagtgtcccagggaaggcgatgctactggtgacaaaggggcttacactcaggcagaggtccttctttccaagtgtgaatgaaggccatgttagcctttctcttgaaaaggccctttcctcatctgtaactggggag

SEQ ID NO: 55 - DNA, 2231 bp, synthetic construct; identical to SEQ ID NO: 54
  source 1..2231: mol_type = other DNA

SEQ ID NO: 56 - DNA, 2301 bp, synthetic construct
  source 1..2301: mol_type = other DNA
atctcatttgaccatcatttgacctattgtctccctgtgggtaggcctcagagccacacacctcaggccaggagtaccattcatccagacgtgaacatcttcccgaggcttccagagttcttggttcacaccggggctaacatggctgggcttctgctgcagtggcaggagctctgtgcacagagaacagcctcatctgctcgccttgtttccacctcccctcccattgccccaggttctttggccccacagcggccacatctgccgttggtgccaataggttttccaggagctggttgaggtgggagggagggagagggttgtgatcaggctgaggcatggggattggatatagtctccgtgtcatgatttatttggtcagtcagtcctagtgcgaccctggggtaatggggatgtgttctcgtcacgttgggcctggctgaccagctttatctcttggcacagaggcaggcagcggcgctaccaatttttctttgttgaagcaggccggggatgtggaggaaaatccggggccaatggctcttcctgtgactgcccttctgctgcccctggctctcctgctccatgctgcccggccagacatccagatgacacagacaaccagcagcctcagcgccagcctgggggacagagtgaccattagctgccgggcctctcaggacatcagcaaatacctgaactggtaccagcagaaaccagatggcactgtcaagctgctgatttaccacacctccaggctccacagcggcgtgcccagtcgcttcagcggcagtgggagcgggacagattattccctcacaatctccaacctggagcaggaagatattgccacatacttctgccagcaaggcaacaccctgccatacacatttggaggcggcaccaaattggagatcaccggcggtggtggatctggaggagggggcagcggaggtggcggctctgaggtgaaactgcaggagagtggccctggcctggtggctcccagccagagcctttctgtcacctgcaccgtgtctggggtgtccctgcctgactatggagtctcctggatccggcagcctccaagaaaaggactggaatggctgggcgtcatctggggaagtgagaccacctactataattcagccctcaagtcccggctcaccatcattaaggacaactccaaatcccaggtgttcctgaagatgaattctctccagactgatgacacagccatctactactgtgccaagcattattattacggcgggtcctatgccatggactactggggccaggggaccagtgtcactgtttcttctgaaagcaagtatggccccccatgccctccctgccccggacagccgcgggagccccaggtctacaccctcccaccctccagagatgagctgaccaagaaccaggtttcactgacatgcctggtgaagggcttctacccctctgacattgctgtggagtgggagagcaatgggcagccagagaacaactacaagaccacacctcctgtcctggacagcgacggctccttcttcctctacagtaagctcactgtggacaagagccgctggcagcagggcaatgtcttctcctgcagcgtgatgcacgaggccctgcacaatgcctatacccagaagtcactctctctgagccctggaaagaaggatcccaagttttgggtcctcgtggtggtcgggggtgtgctggcctgctacagcttgctggtcacagtggccttcatcatcttctgggtgcgctccaagaggagccggctgcttcacagtgattacatgaacatgacccccaggaggccaggacccaccaggaagcactaccagccctacgctcccccgcgggactttgctgcttaccgcagcagagtgaaggtgggtaccactgcgctttgcgaggagggcacggggtcccccacttgatggatgttcagaggggccttggtcttggaaggtctcaagctcgggtggtgcctggggcttggtatccaggagcaaagcaaggaccagccaagtgtgtgccttgagtgggctgaggaggaggtggcagtgtctggctgagatggacagggtaggagggagagcctggtgctaggcacctccatgacaagccgtacaaatgtgtgcacatcagagtgtcccagggaaggcgatgctactggtgacaaaggggcttacactcaggcagaggtccttctttccaagtgtgaatgaaggccatgttagcctttctcttgaaaaggccctttcctcatctgtaactggggag

SEQ ID NO: 57 - DNA, 2301 bp, synthetic construct; identical to SEQ ID NO: 56
  source 1..2301: mol_type = other DNA

SEQ ID NO: 58 - DNA, 2231 bp, synthetic construct
  source 1..2231: mol_type = other DNA
acaccggggctaacatggctgggcttctgctgcagtggcaggagctctgtgcacagagaacagcctcatctgctcgccttgtttccacctcccctcccattgccccaggttctttggccccacagcggccacatctgccgttggtgccaataggttttccaggagctggttgaggtgggagggagggagagggttgtgatcaggctgaggcatggggattggatatagtctccgtgtcatgatttatttggtcagtcagtcctagtgccaccctggggtaatggggatgtgttctcgtcaccttgggcctggctgaccagctttatctcttggcacagaggcacagagctttggcctgctggatcccaaactctgctacctgctggatggaatcctcttcggcagcggcgctaccaatttttctttgttgaagcaggccggggatgtggaggaaaatccggggccaatggctcttcctgtgactgcccttctgctgcccctggctctcctgctccatgctgcccggccagacatccagatgacacagacaaccagcagcctcagcgccagcctgggggacagagtgaccattagctgccgggcctctcaggacatcagcaaatacctgaactggtaccagcagaaaccagatggcactgtcaagctgctgatttaccacacctccaggctccacagcggcgtgcccagtcgcttcagcggcagtgggagcgggacagattattccctcacaatctccaacctggagcaggaagatattgccacatacttctgccagcaaggcaacaccctgccatacacatttggaggcggcaccaaattggagatcaccggcggtggtggatctggaggagggggcagcggaggtggcggctctgaggtgaaactgcaggagagtggccctggcctggtggctcccagccagagcctttctgtcacctgcaccgtgtctggggtgtccctgcctgactatggagtctcctggatccggcagcctccaagaaaaggactggaatggctgggcgtcatctggggaagtgagaccacctactataattcagccctcaagtcccggctcaccatcattaaggacaactccaaatcccaggtgttcctgaagatgaattctctccagactgatgacacagccatctactactgtgccaagcattattattacggcgggtcctatgccatggactactggggccaggggaccagtgtcactgtttcttctgaaagcaagtatggccccccatgccctccctgccccggacagccgcgggagccccaggtctacaccctcccaccctccagagatgagctgaccaagaaccaggtttcactgacatgcctggtgaagggcttctacccctctgacattgctgtggagtgggagagcaatgggcagccagagaacaactacaagaccacacctcctgtcctggacagcgacggctccttcttcctctacagtaagctcactgtggacaagagccgctggcagcagggcaatgtcttctcctgcagcgtgatgcacgaggccctgcacaatgcctatacccagaagtcactctctctgagccctggaaagaaggatcccaagttttgggtcctcgtggtggtcgggggtgtgctggcctgctacagcttgctggtcacagtggccttcatcatcttctgggtgcgctccaagaggagccggctgcttcacagtgattacatgaacatgacccccaggaggccaggacccaccaggaagcactaccagccctacgctcccccgcgggactttgctgcttaccgcagcagagtgaaggtgggtaccactgggctttgggaggagggcacggggtcccccacttgatggatgttcagaggggccttggtcttggaaggtctcaagctcgggtggtgcctggggcttggtatccaggagcaaagcaaggaccagccaagtgtgtgccttgagtgggctgaggaggaggtggcagtgtctggctgagatggacagggtaggagggagagcctggtgctaggcacctccatgacaagccgtacaaatgtgtgcacatcagagtgtcccagggaaggcgatgctactggtgacaaaggggcttacactcaggcagaggtccttctttccaagtgtgaatgaaggccatgttagcctttctcttgaaaaggccctttcctcatctgtaactggggag

SEQ ID NO: 59 - DNA, 2301 bp, synthetic construct; identical to SEQ ID NO: 56
  source 1..2301: mol_type = other DNA

SEQ ID NO: 60 - DNA, 2301 bp, synthetic construct; identical to SEQ ID NO: 56
  source 1..2301: mol_type = other DNA

SEQ ID NO: 61 - DNA, 2138 bp, synthetic construct
  source 1..2138: mol_type = other DNA
aagctcatttggccagagtggaaatggaattgggagaaatcgatgaccaaatgtaaacacttggtgcctgatatagcttgacaccaagttagccccaagtgaaataccctggcaatattaatgtgtcttttcccgatattcctcaggtactccaaagattcaggtttactcacgtcatccagcagagaatggaaagtcaaatttcctgaattgctatgtgtctgggtttcatccatccgacattgaagttgacttactgaagaatggagagagaattgaaaaagtggagcattcagacttgtctttcagcaaggactggtctttctatctcttgtactacactgaattcacccccactgaaaaagatgagtatgcttgcagggttaaccatgtcacattgtcacaacctaaaattgtgaaatgggacagggacatgggtgggggcggatcaggcggcggcggttctgggggaggcggctcaggtggcggtgggagtggatcccattccctgaagtatttccacaccagcgttagtcggccgggaaggggagaaccaagattcatttccgtcggctatgtcgacgatacccaatttgtgcgatttgataatgacgcagcttcaccccgcatggtgcctcgggctccttggatggagcaagaaggctcagagtactgggaccgggagacccgatctgcgcgcgatacagcacaaatctttagggtcaaccttcgaacattgaggggctactacaaccagagtgaggcaggttcccatacgttgcaatggatgcatggttgcgaacttggtccagatgggaggttcctcagaggttatgaacaatttgcttacgatggaaaggactaccttacactcaatgaggacctccgcagctggaccgccgttgacaccgctgctcaaatctccgagcaaaagagtaatgacgcgtcagaagcggagcatcagcgcgcctacctcgaggacacgtgcgttgagtggctccataaatacctggaaaaagggaaagaaaccctcctccacctggagccaccgaagacccacgtcacgcatcacccaatatccgatcacgaggctacactgaggtgctgggctctcggtttctatccggcagaaataaccctgacctggcagcaggatggtgagggccatacgcaggacacggagcttgtcgagactcgacccgccggtgatggaacattccaaaaatgggctgctgtcgttgtaccctctggagaagaacaacgatacacctgccacgtgcagcatgagggactgccggaaccggtaaccttgcgctggaagccggcgtcacaaccaacgatacccatcgtcggcattatagccggacttgttctcctgggaagcgtggtcagcggagctgtcgtagcggccgtaatttggaggaaaaagtcttctgggggaaagggtgggtcatactctaaagcggagtggtctgactcagcacagggttccgaatcccactccctgtgagcggccgcgtcgagtctagagggcccgtttaaacccgctgatcagcctcgactgtgccttctagttgccagccatctgttgtttgcccctcccccgtgccttccttgaccctggaaggtgccactcccactgtcctttcctaataaaatgaggaaattgcatcgcattgtctgagtaggtgtcattctattctggggggtggggtggggcaggacagcaagggggaggattgggaagacaatagcaggcatgctggggatgcggtgggctctatggccaagatagttaagtggggtaagtcttacattcttttgtaagctgctgaaagttgtgtatgagtagtcatatcataaagctgctttgatataaaaaaggtctatggccatactaccctgaatgagtcccatcccatctgatataaacaatctgcatattgggattgtcagggaatgttcttaaagatcagattagtggcacctgctgagatactgatgcacagcatggtttctgaaccagtagtttccctgcagttgagcagggagcagcagcagcacttgcacaaatacatatacactcttaacacttcttacctactggcttcctctagcttttgtggcagcttcaggta

SEQ ID NO: 62 - DNA, 2173 bp, synthetic construct
  source 1..2173: mol_type = other DNA
aagctcatttggccagagtggaaatggaattgggagaaatcgatgaccaaatgtaaacacttggtgcctgatatagcttgacaccaagttagccccaagtgaaataccctggcaatattaatgtgtcttttcccgatattcctcaggtactccaaagattcaggtttactcacgtcatccagcagagaatggaaagtcaaatttcctgaattgctatgtgtctgggtttcatccatccgacattgaagttgacttactgaagaatggagagagaattgaaaaagtggagcattcagacttgtctttcagcaaggactggtctttctatctcttgtactacactgaattcacccccactgaaaaagatgagtatgcctgccgtgtgaaccatgtgactttgtcacagcccaagattgtgaaatgggacagggacatgggtgggggcggatcaggcggcggcggttctgggggaggcggctcaggtggcggtgggagtggatcccattccctgaagtatttccacaccagcgttagtcggccgggaaggggagaaccaagattcatttccgtcggctatgtcgacgatacccaatttgtgcgatttgataatgacgcagcttcaccccgcatggtgcctcgggctccttggatggagcaagaaggctcagagtactgggaccgggagacccgatctgcgcgcgatacagcacaaatctttagggtcaaccttcgaacattgaggggctactacaaccagagtgaggcaggttcccatacgttgcaatggatgcatggttgcgaacttggtccagatgggaggttcctcagaggttatgaacaatttgcttacgatggaaaggactaccttacactcaatgaggacctccgcagctggaccgccgttgacaccgctgctcaaatctccgagcaaaagagtaatgacgcgtcagaagcggagcatcagcgcgcctacctcgaggacacgtgcgttgagtggctccataaatacctggaaaaagggaaagaaaccctcctccacctggagccaccgaagacccacgtcacgcatcacccaatatccgatcacgaggctacactgaggtgctgggctctcggtttctatccggcagaaataaccctgacctggcagcaggatggtgagggccatacgcaggacacggagcttgtcgagactcgacccgccggtgatggaacattccaaaaatgggctgctgtcgttgtaccctctggagaagaacaacgatacacctgccacgtgcagcatgagggactgccggaaccggtaaccttgcgctggaagccggcgtcacaaccaacgatacccatcgtcggcattatagccggacttgttctcctgggaagcgtggtcagcggagctgtcgtagcggccgtaatttggaggaaaaagtcttctgggggaaagggtgggtcatactctaaagcggagtggtctgactcagcacagggttccgaatcccactccctgtgagcggccgcgtcgagtctagagggcccgtttaaacccgctgatcagcctcgactgtgccttctagttgccagccatctgttgtttgcccctcccccgtgccttccttgaccctggaaggtgccactcccactgtcctttcctaataaaatgaggaaattgcatcgcattgtctgagtaggtgtcattctattctggggggtggggtggggcaggacagcaagggggaggattgggaagacaatagcaggcatgctggggatgcggtgggctctatggaaaaggtctatggccatactaccctgaatgagtcccatcccatctgatataaacaatctgcatattgggattgtcagggaatgttcttaaagatcagattagtggcacctgctgagatactgatgcacagcatggtttctgaaccagtagtttccctgcagttgagcagggagcagcagcagcacttgcacaaatacatatacactcttaacacttcttacctactggcttcctctagcttttgtggcagcttcaggtatatttagcactgaacgaacatctcaagaaggtataggcctttgtttgtaagtcctgctgtcctagcatcctataatcctggacttctccagtactttctggctggattggtatctgaggctagtagga

SEQ ID NO: 63 - DNA, 2173 bp, synthetic construct
  source 1..2173: mol_type = other DNA
aagctcatttggccagagtggaaatggaattgggagaaatcgatgaccaaatgtaaacacttggtgcctgatatagcttgacaccaagttagccccaagtgaaataccctggcaatattaatgtgtcttttcccgatattcctcaggtactccaaagattcaggtttactcacgtcatccagcagagaatggaaagtcaaatttcctgaattgctatgtgtctgggtttcatccatccgacattgaagttgacttactgaagaatggagagagaattgaaaaagtggagcattcagacttgtctttcagcaaggactggtctttctatctcttgtactacactgaattcacccccactgaaaaagatgagtatgcatgccgtgtgaaccatgtgactttgtcacagcctaaaattgtgaaatgggacagggacatgggtgggggcggatcaggcggcggcggttctgggggaggcggctcaggtggcggtgggagtggatcccattccctgaagtatttccacaccagcgttagtcggccgggaaggggagaaccaagattcatttccgtcggctatgtcgacgatacccaatttgtgcgatttgataatgacgcagcttcaccccgcatggtgcctcgggctccttggatggagcaagaaggctcagagtactgggaccgggagacccgatctgcgcgcgatacagcacaaatctttagggtcaaccttcgaacattgaggggctactacaaccagagtgaggcaggttcccatacgttgcaatggatgcatggttgcgaacttggtccagatgggaggttcctcagaggttatgaacaatttgcttacgatggaaaggactaccttacactcaatgaggacctccgcagctggaccgccgttgacaccgctgctcaaatctccgagcaaaagagtaatgacgcgtcagaagcggagcatcagcgcgcctacctcgaggacacgtgcgttgagtggctccataaatacctggaaaaagggaaagaaaccctcctccacctggagccaccgaagacccacgtcacgcatcacccaatatccgatcacgaggctacactgaggtgctgggctctcggtttctatccggcagaaataaccctgacctggcagcaggatggtgagggccatacgcaggacacggagcttgtcgagactcgacccgccggtgatggaacattccaaaaatgggctgctgtcgttgtaccctctggagaagaacaacgatacacctgccacgtgcagcatgagggactgccggaaccggtaaccttgcgctggaagccggcgtcacaaccaacgatacccatcgtcggcattatagccggacttgttctcctgggaagcgtggtcagcggagctgtcgtagcggccgtaatttggaggaaaaagtcttctgggggaaagggtgggtcatactctaaagcggagtggtctgactcagcacagggttccgaatcccactccctgtgagcggccgcgtcgagtctagagggcccgtttaaacccgctgatcagcctcgactgtgccttctagttgccagccatctgttgtttgcccctcccccgtgccttccttgaccctggaaggtgccactcccactgtcctttcctaataaaatgaggaaattgcatcgcattgtctgagtaggtgtcattctattctggggggtggggtggggcaggacagcaagggggaggattgggaagacaatagcaggcatgctggggatgcggtgggctctatggaaaaggtctatggccatactaccctgaatgagtcccatcccatctgatataaacaatctgcatattgggattgtcagggaatgttcttaaagatcagattagtggcacctgctgagatactgatgcacagcatggtttctgaaccagtagtttccctgcagttgagcagggagcagcagcagcacttgcacaaatacatatacactcttaacacttcttacctactggcttcctctagcttttgtggcagcttcaggtatatttagcactgaacgaacatctcaagaaggtataggcctttgtttgtaagtcctgctgtcctagcatcctataatcctggacttctccagtactttctggctggattggtatctgaggctagtagga

SEQ ID NO: 64 - DNA, 2138 bp, synthetic construct; identical to SEQ ID NO: 61
  source 1..2138: mol_type = other DNA

SEQ ID NO: 65 - DNA, 2138 bp, synthetic construct; identical to SEQ ID NO: 61
  source 1..2138: mol_type = other DNA